European Patent Application EP 4 410 371 A1, published August 7, 2024. Title: Therapeutic VHH antibodies against alpha-hemolysin from Staphylococcus aureus. Applicant: Max-Planck-Gesellschaft zur Foerderung der Wissenschaften e.V. The sequence listing filed with the application follows.

SEQUENCE LISTING (70 sequences)

SEQ ID NO: 1 - protein, 293 aa, synthetic construct
  REGION 1..293: note = HLA used for hemolysis assays and crystallization
ADSDINIKTGTTDIGSNTTVKTGDLVTYDKENGMHKKVFYSFIDDKNHNKKLLVIRTKGTIAGQYRVYSEEGANKSGLAWPSAFKVQLQLPDNEVAQISDYYPRNSIDTKEYMSTLTYGFNGNVTGDDTGKIGGLIGANVSIGHTLKYVQPDFKTILESPTDKKVGWKVIFNNMVNQNWGPYDRDSWNPVYGNQLFMKTRNGSMKAADNFLDPNKASSLLSSGFSPDFATVITMDRKASKQQTNIDVIYERVRDDYQLHWTSTNWKGTNTKDKWTDRSSERYKIDWEKEEMTN

SEQ ID NO: 2 - protein, 300 aa, synthetic construct
  REGION 1..300: note = Cys-HLA used for Octet assays
SECGSSGADSDINIKTGTTDIGSNTTVKTGDLVTYDKENGMHKKVFYSFIDDKNHNKKLLVIRTKGTIAGQYRVYSEEGANKSGLAWPSAFKVQLQLPDNEVAQISDYYPRNSIDTKEYMSTLTYGFNGNVTGDDTGKIGGLIGANVSIGHTLKYVQPDFKTILESPTDKKVGWKVIFNNMVNQNWGPYDRDSWNPVYGNQLFMKTRNGSMKAADNFLDPNKASSLLSSGFSPDFATVITMDRKASKQQTNIDVIYERVRDDYQLHWTSTNWKGTNTKDKWTDRSSERYKIDWEKEEMTN

SEQ ID NO: 3 - protein, 123 aa, synthetic construct
  REGION 1..123: note = VHH antibody sequence Ma7A07
QVQLVESGGGLVQPGGSLRLSCAASGFTLGDYTLGWFRQAPGKQREGVSSIASSALSIYIADSVKGRFTISRDDAKNTIYLHMNNLKPEDTGVYYCARGVDSWRWVPSAMDLWGKGTLVTVSS

SEQ ID NO: 4 - protein, 11 aa, synthetic construct
  REGION 1..11: note = CDR1_Ma7A07
SGFTLGDYTLG

SEQ ID NO: 5 - protein, 15 aa, synthetic construct
  REGION 1..15: note = CDR2_Ma7A07
SSIASSALSIYIADS

SEQ ID NO: 6 - protein, 16 aa, synthetic construct
  REGION 1..16: note = CDR3_Ma7A07
RGVDSWRWVPSAMDLW

SEQ ID NO: 7 - protein, 123 aa, synthetic construct
  REGION 1..123: note = VHH antibody sequence Ma7A08
QVQLVESGGGLVQPGGSLTLSCAASGFTLGDYTLGWFRQAPGKQREGVSSIASSVLSVYIADSVKGRFTISRDDAKNTIYLHMNNLKPEDTGVYYCARGVDSWRWVPSAMDLWGKGTLVTVSS

SEQ ID NO: 8 - protein, 11 aa, synthetic construct
  REGION 1..11: note = CDR1_Ma7A08
SGFTLGDYTLG

SEQ ID NO: 9 - protein, 15 aa, synthetic construct
  REGION 1..15: note = CDR2_Ma7A08
SSIASSVLSVYIADS

SEQ ID NO: 10 - protein, 16 aa, synthetic construct
  REGION 1..16: note = CDR3_Ma7A08
RGVDSWRWVPSAMDLW

SEQ ID NO: 11 - protein, 123 aa, unidentified
  REGION 1..123: note = VHH antibody sequence Ma7B03
QVQLVESGGGLVQPGGSLRLSCAASGFTLSNYYVGWFRQAPGKQREGVSSIGSSDLSIYIADSVKGRFTISRDNAKNTIYLHMNNLKPDDTGVYYCARGTDSWRWVPSAMDLWGKGTQVTVSS

SEQ ID NO: 12 - protein, 11 aa, synthetic construct
  REGION 1..11: note = CDR1_Ma7B03
SGFTLSNYYVG

SEQ ID NO: 13 - protein, 15 aa, synthetic construct
  REGION 1..15: note = CDR2_Ma7B03
SSIGSSDLSIYIADS

SEQ ID NO: 14 - protein, 16 aa, synthetic construct
  REGION 1..16: note = CDR3_Ma7B03
RGTDSWRWVPSAMDLW

SEQ ID NO: 15 - protein, 132 aa, synthetic construct
  REGION 1..132: note = VHH antibody sequence Ma7B12
QVQLVESGGGLVQPGGSLRLSCAASGFTLGDYTLGWFRQAPGKQREGVSSIASSALSIYIADSVKGRFTISRDNAKNTVYLHMNNLKPEDTGVYYCARGIDNWRWVPSAMDLWGKGTQVTVSSGKTLVTVSS

SEQ ID NO: 16 - protein, 11 aa, synthetic construct
  REGION 1..11: note = CDR1_Ma7B12
SGFTLGDYTLG

SEQ ID NO: 17 - protein, 15 aa, synthetic construct
  REGION 1..15: note = CDR2_Ma7B12
SSIASSALSIYIADS

SEQ ID NO: 18 - protein, 16 aa, synthetic construct
  REGION 1..16: note = CDR3_Ma7B12
RGIDNWRWVPSAMDLW

SEQ ID NO: 19 - protein, 125 aa, synthetic construct
  REGION 1..125: note = VHH antibody sequence Ma7B01
QVQLVESGGGLVQAGDSLSLSCAASGRTFSNYAMGWFRQAPGKERHFVAVINQIGDSTWYPDFAKGRFTISRDNAKNTLYLQMNSLKPEDTAVYYCAATDPRSYWRIWPHEYGYWGQGTQVTVSS

SEQ ID NO: 20 - protein, 11 aa, synthetic construct
  REGION 1..11: note = CDR1_Ma7B01
SGRTFSNYAMG

SEQ ID NO: 21 - protein, 15 aa, synthetic construct
  REGION 1..15: note = CDR2_Ma7B01
AVINQIGDSTWYPDF

SEQ ID NO: 22 - protein, 18 aa, synthetic construct
  REGION 1..18: note = CDR3_Ma7B01
ATDPRSYWRIWPHEYGYW

SEQ ID NO: 23 - protein, 125 aa, synthetic construct
  REGION 1..125: note = VHH antibody sequence Ma7C02
QVQLVESGGGLVQAGGSLRLSCAASGRTFSDYAMGWFRQAAGKDRDFVAVITRSGDSTYYPDSTKGRFTISRDNAKNTMYLQMNSLKPEDTARYYCAATDPTNYWRIWEHEFDYWGQGTQVTVSS

SEQ ID NO: 24 - protein, 11 aa, synthetic construct
  REGION 1..11: note = CDR1_Ma7C02
SGRTFSDYAMG

SEQ ID NO: 25 - protein, 15 aa, synthetic construct
  REGION 1..15: note = CDR2_Ma7C02
AVITRSGDSTYYPDS

SEQ ID NO: 26 - protein, 18 aa, synthetic construct
  REGION 1..18: note = CDR3_Ma7C02
ATDPTNYWRIWEHEFDYW

SEQ ID NO: 27 - protein, 125 aa, synthetic construct
  REGION 1..125: note = VHH antibody sequence Ma7E01
QVQLVESGGGSVQAGDSLSLSCVASERTFSNYAMGWFRQAPGKERHFVAVINPIGEETWYPDFAKGRFTISRDNAKNTLYLQMNSLKPEDTAVYYCAATDPRSYWRIWEHEFDYWGQGTQVTVSS

SEQ ID NO: 28 - protein, 11 aa, synthetic construct
  REGION 1..11: note = CDR1_Ma7E01
SERTFSNYAMG

SEQ ID NO: 29 - protein, 15 aa, synthetic construct
  REGION 1..15: note = CDR2_Ma7E01
AVINPIGEETWYPDF

SEQ ID NO: 30 - protein, 18 aa, synthetic construct
  REGION 1..18: note = CDR3_Ma7E01
ATDPRSYWRIWEHEFDYW

SEQ ID NO: 31 - protein, 126 aa, synthetic construct
  REGION 1..126: note = VHH antibody sequence Ma7F02
QVQLVESGGGLVQAGGSLRLSCTVSGSIDSLHTMGWFRQAPGKKRDFVAVVSWSGGNTYYPDYAKGRFTISRDNTKNTVYLQMNSLKPEDTAIYYCAAESGSGNYWKIWEHEFDSWGQGTQVTVSS

SEQ ID NO: 32 - protein, 11 aa, synthetic construct
  REGION 1..11: note = CDR1_ Ma7F02
SGSIDSLHTMG

SEQ ID NO: 33 - protein, 15 aa, synthetic construct
  REGION 1..15: note = CDR2_Ma7F02
AVVSWSGGNTYYPDY

SEQ ID NO: 34 - protein, 19 aa, synthetic construct
  REGION 1..19: note = CDR3_Ma7F02
AESGSGNYWKIWEHEFDSW

SEQ ID NO: 35 - protein, 126 aa, synthetic construct
  REGION 1..126: note = VHH antibody sequence Ma7D06
QVQLVESGGGLVQAGGSLRLSCAASGSISGIDTMAWFRQIPGKDREFVAVIKWAAGSTWYPDFVKGRFTVSRDNAKNMVYLQMDSVKPEDTAIYYCAAAAGEKYYYRLFPYEYDYWGQGTQVTVSS

SEQ ID NO: 36 - protein, 11 aa, synthetic construct
  REGION 1..11: note = CDR1_Ma7D06
SGSISGIDTMA

SEQ ID NO: 37 - protein, 15 aa, synthetic construct
  REGION 1..15: note = CDR2_Ma7D06
AVIKWAAGSTWYPDF

SEQ ID NO: 38 - protein, 19 aa, synthetic construct
  REGION 1..19: note = CDR3_Ma7D06
AAAGEKYYYRLFPYEYDYW

SEQ ID NO: 39 - protein, 124 aa, synthetic construct
  REGION 1..124: note = VHH antibody sequence Ma7C11
QVQLVESGGGLVRAGGSLRLSCAASGSISSVNGMGWFRQAPGKERLFVAQVSLLDSSTYYADSVKGRFTISRDDAKNTMYLQMNNVRPEETAVYYCAATKLRIGTAFSSEYDYWGQGTQVTVSS

SEQ ID NO: 40 - protein, 11 aa, synthetic construct
  REGION 1..11: note = CDR1_Ma7C11
SGSISSVNGMG

SEQ ID NO: 41 - protein, 15 aa, synthetic construct
  REGION 1..15: note = CDR2_Ma7C11
AQVSLLDSSTYYADS

SEQ ID NO: 42 - protein, 17 aa, synthetic construct
  REGION 1..17: note = CDR3_Ma7C11
ATKLRIGTAFSSEYDYW

SEQ ID NO: 43 - protein, 126 aa, synthetic construct
  REGION 1..126: note = VHH antibody sequence Ma8E03
QVQLVESGGGLVHPGGSLRLSCAASGSSLDHYVIGWFRQVPGKEREGVSCISRSGGSTNYADSVKGRFTVSRDNVKNMVYLQMNSLEPEDSAEYYCAAQRNLGNFCVLGWLEYDDWGQGTQVTVSS

SEQ ID NO: 44 - protein, 11 aa, synthetic construct
  REGION 1..11: note = CDR1_Ma8E03
SGSSLDHYVIG

SEQ ID NO: 45 - protein, 15 aa, synthetic construct
  REGION 1..15: note = CDR2_Ma8E03
SCISRSGGSTNYADS

SEQ ID NO: 46 - protein, 19 aa, synthetic construct
  REGION 1..19: note = CDR3_Ma8E03
AQRNLGNFCVLGWLEYDDW

SEQ ID NO: 47 - protein, 126 aa, synthetic construct
  REGION 1..126: note = VHH antibody sequence Ma8G02
QVQLVESGGGLVLPGGSLRLSCAASGSSLDHYVIGWFRQYPGKEREGVSCISRSGGSTNYADSVKGRFTVSRDNVKNMVYLQMNSLEPEDSAEYYCAAQRNLGNFCVLGWVEYDDWGQGTQVTVSS

SEQ ID NO: 48 - protein, 11 aa, synthetic construct
  REGION 1..11: note = CDR1_Ma8G02
SGSSLDHYVIG

SEQ ID NO: 49 - protein, 15 aa, synthetic construct
  REGION 1..15: note = CDR2_Ma8G02
SCISRSGGSTNYADS

SEQ ID NO: 50 - protein, 19 aa, synthetic construct
  REGION 1..19: note = CDR3_Ma8G02
AQRNLGNFCVLGWVEYDDW

SEQ ID NO: 51 - protein, 125 aa, synthetic construct
  REGION 1..125: note = VHH antibody sequence Ma8H03
QVQLVESGGGLVHPGGSLRLSCAASGSSLDHYVIGWFRQVPGKQREGISCISSGGSTNYADSVKGRFTVSRDNVKSTVYLQMNSLAPDDSAEYYCAAQRNLGNFCVLGWLEYDDWGQGTQVTVSS

SEQ ID NO: 52 - protein, 11 aa, synthetic construct
  REGION 1..11: note = CDR1_Ma8H03
SGSSLDHYVIG

SEQ ID NO: 53 - protein, 14 aa, synthetic construct
  REGION 1..14: note = CDR2_Ma8H03
SCISSGGSTNYADS

SEQ ID NO: 54 - protein, 19 aa, synthetic construct
  REGION 1..19: note = CDR3_Ma8H03
AQRNLGNFCVLGWLEYDDW

SEQ ID NO: 55 - protein, 126 aa, synthetic construct
  REGION 1..126: note = VHH antibody sequence Ma8A05
QVQLVESGGGLVQPGGSLRLSCAASPASGFTLDLYTIAWFLQAPGKEREGVSAISLSDEITYYSDAVKGRFTISRDSAKNTVFLQMDRLKPEDTGVYYCAIGAFDFILKEADADYWGQGTQVTVSS

SEQ ID NO: 56 - protein, 14 aa, synthetic construct
  REGION 1..14: note = CDR1_Ma8A05
SPASGFTLDLYTIA

SEQ ID NO: 57 - protein, 15 aa, synthetic construct
  REGION 1..15: note = CDR2_Ma8A05
SAISLSDEITYYSDA

SEQ ID NO: 58 - protein, 16 aa, synthetic construct
  REGION 1..16: note = CDR3_Ma8A05
IGAFDFILKEADADYW

SEQ ID NO: 59 - protein, 126 aa, synthetic construct
  REGION 1..126: note = VHH antibody sequence Ma8D05
QVQLVESGGGLVQPGGSLRLSCAASPASGFTLDLYTIAWFLQAPGKEREGVSAISLSDEITYYSDTVKGRFTISRDSAKNTVFLQMDRLKPEDTGVYYCAIGAFDFILKEADADYWGQGTQVTVSS

SEQ ID NO: 60 - protein, 14 aa, synthetic construct
  REGION 1..14: note = CDR1_Ma8D05
SPASGFTLDLYTIA

SEQ ID NO: 61 - protein, 15 aa, synthetic construct
  REGION 1..15: note = CDR2_Ma8D05
SAISLSDEITYYSDT

SEQ ID NO: 62 - protein, 16 aa, synthetic construct
  REGION 1..16: note = CDR3_Ma8D05
IGAFDFILKEADADYW

SEQ ID NO: 63 - protein, 117 aa, synthetic construct
  REGION 1..117: note = VHH antibody sequence Ma8D07
QVQLVESGGGLVQPGGSLRLSCAASESIYKLNAMGWYRQAPGKELELVTTISSGGSTFYTDPVKGRFTISTDNAKNTVYLQMRSLKPEDTAMYYCAANPTYNHYSARGQGTQVTVSS

SEQ ID NO: 64 - protein, 11 aa, synthetic construct
  REGION 1..11: note = CDR1_Ma8D07
SESIYKLNAMG

SEQ ID NO: 65 - protein, 14 aa, synthetic construct
  REGION 1..14: note = CDR2_Ma8D07
TTISSGGSTFYTDP

SEQ ID NO: 66 - protein, 11 aa, synthetic construct
  REGION 1..11: note = CDR3_Ma8D07
ANPTYNHYSAR

SEQ ID NO: 67 - protein, 117 aa, synthetic construct
  REGION 1..117: note = VHH antibody sequence Ma8D08
QVQLVESGGGFVQAGGSLRLSCAASESIYKLNAMGWYRQAPGKELELVTTISSGGSTFYTDPVKGRFTISTDNAKNTVYLQMRSLKPEDTAMYYCAANPTYNHYSARGQGTQVTVSS

SEQ ID NO: 68 - protein, 11 aa, synthetic construct
  REGION 1..11: note = CDR1_Ma8D08
SESIYKLNAMG

SEQ ID NO: 69 - protein, 14 aa, synthetic construct
  REGION 1..14: note = CDR2_Ma8D08
TTISSGGSTFYTDP

SEQ ID NO: 70 - protein, 11 aa, synthetic construct
  REGION 1..11: note = CDR3_Ma8D08
ANPTYNHYSAR